European Patent Specification EP 3 181 581 B1, published September 25, 2024. Title: Antibodies with modified affinity to FCRN that promote antigen clearance. Applicant: CHUGAI SEIYAKU KABUSHIKI KAISHA. The sequence listing filed with the application follows.

SEQUENCE LISTING (31 sequences)

SEQ ID NO: 1 - protein, 447 aa, Artificial
  An artificially synthesized peptide sequence
QVQLQESGPGLVKPSETLSLTCAVSGYSISDDQAWSWVRQPPGEGLEWIGYISYSGITNYNPSLKGRVTISRDTSKNQFSLKLSSVTAADTAAYYCARSLARTTAMDYWGEGTLVTVSSASTKGPSVFPLAPSSKSTSGGTAALGCLVKDYFPEPVTVSWNSGALTSGVHTFPAVLQSSGLYSLSSVVTVPSSSLGTQTYICNVNHKPSNTKVDKKVEPKSCDKTHTCPPCPAPELLGGPSVFLFPPKPKDTLMISRTPEVTCVVVDVSHEDPEVKFNWYVDGVEVHNAKTKPREEQYNSTYRVVSVLTVLHQDWLNGKEYKCKVSNKALPAPIEKTISKAKGQPREPQVYTLPPSRDELTKNQVSLTCLVKGFYPSDIAVEWESNGQPENNYKTTPPVLDSDGSFFLYSKLTVDKSRWQQGNVFSCSVMHEALHNHYTQKSLSLSP

SEQ ID NO: 2 - protein, 214 aa, Artificial
  An artificially synthesized peptide sequence
DIQMTQSPSSLSASVGDSVTITCQASQDISSYLNWYQQKPGKAPELLIYYGSELHSGVPSRFSGSGSGTDFTFTISSLEAEDAATYYCQQGNSLPYTFGQGTKVEIERTVAAPSVFIFPPSDEQLKSGTASVVCLLNNFYPREAKVQWKVDNALQSGNSQESVTEQDSKDSTYSLSSTLTLSKADYEKHKVYACEVTHQGLSSPVTKSFNRGEC

SEQ ID NO: 3 - protein, 447 aa, Artificial
  An artificially synthesized peptide sequence
QVQLQESGPGLVKPSETLSLTCAVSGYSISDDQAWSWVRQPPGEGLEWIGYISYSGITNYNPSLKGRVTISRDTSKNQFSLKLSSVTAADTAAYYCARSLARTTAMDYWGEGTLVTVSSASTKGPSVFPLAPSSKSTSGGTAALGCLVKDYFPEPVTVSWNSGALTSGVHTFPAVLQSSGLYSLSSVVTVPSSSLGTQTYICNVNHKPSNTKVDKKVEPKSCDKTHTCPPCPAPELLGGPSVFLFPPKPKDTLWISRTPEVTCVVVDVSHEDPEVKFNWYVDGVEVHNAKTKPREEQYNSTYRVVSVLTVLHQDWLNGKEYKCKVSNKALPAPIEKTISKAKGQPREPQVYTLPPSRDELTKNQVSLTCLVKGFYPSDIAVEWESNGQPENNYKTTPPVLDSDGSFFLYSKLTVDKSRWQQGNVFSCSVMHEALHWHYTQKSLSLSP

SEQ ID NO: 4 - protein, 449 aa, Homo sapiens
QVQLQESGPGLVRPSQTLSLTCTVSGYSITSDHAWSWVRQPPGRGLEWIGYISYSGITTYNPSLKSRVTMLRDTSKNQFSLRLSSVTAADTAVYYCARSLARTTAMDYWGQGSLVTVSSASTKGPSVFPLAPSSKSTSGGTAALGCLVKDYFPEPVTVSWNSGALTSGVHTFPAVLQSSGLYSLSSVVTVPSSSLGTQTYICNVNHKPSNTKVDKKVEPKSCDKTHTCPPCPAPELLGGPSVFLFPPKPKDTLMISRTPEVTCVVVDVSHEDPEVKFNWYVDGVEVHNAKTKPREEQYNSTYRVVSVLTVLHQDWLNGKEYKCKVSNKALPAPIEKTISKAKGQPREPQVYTLPPSRDELTKNQVSLTCLVKGFYPSDIAVEWESNGQPENNYKTTPPVLDSDGSFFLYSKLTVDKSRWQQGNVFSCSVMHEALHNHYTQKSLSLSPGK

SEQ ID NO: 5 - protein, 214 aa, Homo sapiens [sequence omitted]

SEQ ID NO: 6 - protein, 447 aa, Artificial
  An artificially synthesized peptide sequence
QVQLQESGPGLVKPSETLSLTCAVSGHSISHDHAWSWVRQPPGEGLEWIGFISYSGITNYNPSLQGRVTISRDNSKNTLYLQMNSLRAEDTAVYYCARSLARTTAMDYWGEGTLVTVSSASTKGPSVFPLAPSSKSTSGGTAALGCLVKDYFPEPVTVSWNSGALTSGVHTFPAVLQSSGLYSLSSVVTVPSSSLGTQTYICNVNHKPSNTKVDKKVEPKSCDKTHTCPPCPAPELLGGPSVFLFPPKPKDTLMISRTPEVTCVVVDVSHEDPEVKFNWYVDGVEVHNAKTKPREEQYNSTYRVVSVLTVLHQDWLNGKEYKCKVSNKALPAPIEKTISKAKGQPREPQVYTLPPSRDELTKNQVSLTCLVKGFYPSDIAVEWESNGQPENNYKTTPPVLDSDGSFFLYSKLTVDKSRWQQGNVFSCSVMHEALHNHYTQKSLSLSP

SEQ ID NO: 7 - protein, 214 aa, Artificial
  An artificially synthesized peptide sequence
DIQMTQSPSSLSASVGDSVTITCQASTDISSHLNWYQQKPGKAPELLIYYGSHLLSGVPSRFSGSGSGTDFTFTISSLEAEDAATYYCGQGNRLPYTFGQGTKVEIERTVAAPSVFIFPPSDEQLKSGTASVVCLLNNFYPREAKVQWKVDNALQSGNSQESVTEQDSKDSTYSLSSTLTLSKADYEKHKVYACEVTHQGLSSPVTKSFNRGEC

SEQ ID NO: 8 - protein, 447 aa, Artificial
  An artificially synthesized peptide sequence
QVQLQESGPGLVKPSETLSLTCAVSGHSISHDHAWSWVRQPPGEGLEWIGFISYSGITNYNPSLQGRVTISRDNSKNTLYLQMNSLRAEDTAVYYCARSLARTTAMDYWGEGTLVTVSSASTKGPSVFPLAPSSKSTSGGTAALGCLVKDYFPEPVTVSWNSGALTSGVHTFPAVLQSSGLYSLSSVVTVPSSSLGTQTYICNVNHKPSNTKVDKKVEPKSCDKTHTCPPCPAPELLGGPSVFLFPPKPKDTLYITREPEVTCVVVDVSHEDPEVKFNWYVDGVEVHNAKTKPREEQYNSTYRVVSVLTVLHQDWLNGKEYKCKVSNKALPAPIEKTISKAKGQPREPQVYTLPPSRDELTKNQVSLTCLVKGFYPSDIAVEWESNGQPENNYKTTPPVLDSDGSFFLYSKLTVDKSRWQQGNVFSCSVMHEALHNHYTQKSLSLSP

SEQ ID NO: 9 - protein, 447 aa, Artificial
  An artificially synthesized peptide sequence
QVQLQESGPGLVKPSETLSLTCAVSGHSISHDHAWSWVRQPPGEGLEWIGFISYSGITNYNPSLQGRVTISRDNSKNTLYLQMNSLRAEDTAVYYCARSLARTTAMDYWGEGTLVTVSSASTKGPSVFPLAPSSKSTSGGTAALGCLVKDYFPEPVTVSWNSGALTSGVHTFPAVLQSSGLYSLSSVVTVPSSSLGTQTYICNVNHKPSNTKVDKKVEPKSCDKTHTCPPCPAPELLGGPSVFLFPPKPKDTLMISRTPEVTCVVVDVSHEDPEVKFNWYVDGVEVHNAKTKPREEQYNSTYRVVSVLTVLHQDWLNGKEYKCKVSNKALPAPIEKTISKAKGQPREPQVYTLPPSRDELTKNQVSLTCLVKGFYPSDIAVEWESNGQPENNYKTTPPVLDSDGSFFLYSKLTVDKSRWQQGNVFSCSVMHEALHWHYTQKSLSLSP

SEQ ID NO: 10 - protein, 447 aa, Artificial
  An artificially synthesized peptide sequence
QVQLQESGPGLVKPSETLSLTCAVSGHSISHDHAWSWVRQPPGEGLEWIGFISYSGITNYNPSLQGRVTISRDNSKNTLYLQMNSLRAEDTAVYYCARSLARTTAMDYWGEGTLVTVSSASTKGPSVFPLAPSSKSTSGGTAALGCLVKDYFPEPVTVSWNSGALTSGVHTFPAVLQSSGLYSLSSVVTVPSSSLGTQTYICNVNHKPSNTKVDKKVEPKSCDKTHTCPPCPAPELLGGPSVFLFPPKPKDTLMISRTPEVTCVVVDVSHEDPEVKFNWYVDGVEVHNAKTKPREEQYNSTYRVVSVLTFLHQDWLNGKEYKCKVSNKALPAPIEKTISKAKGQPREPQVYTLPPSRDELTKNQVSLTCLVKGFYPSDIAVEWESNGQPENNYKTTPPVLDSDGSFFLYSKLTVDKSRWQQGNVFSCSVMHEALHYHYTQKSLSLSP

SEQ ID NO: 11 - protein, 324 aa, Artificial
  An artificially synthesized peptide sequence
ASTKGPSVFPLAPCSRSTSESTAALGCLVKDYFPEPVTVSWNSGALTSGVHTFPAVLQSSGLYSLSSVVTVPSSNFGTQTYTCNVDHKPSNTKVDKTVERKCCVECPPCPAPPVAGPSVFLFPPKPKDTLMISRTPEVTCVVVDVSHEDPEVQFNWYVDGVEVHNAKTKPREEQFNSTFRVVSVLTVVHQDWLNGKEYKCKVSNKGLPAPIEKTISKTKGQPREPQVYTLPPSREEMTKNQVSLTCLVKGFYPSDIAVEWESNGQPENNYKTTPPMLDSDGSFFLYSKLTVDKSRWQQGNVFSCSVMHEALHNHYTQKSLSLSP

SEQ ID NO: 12 - protein, 324 aa, Artificial
  An artificially synthesized peptide sequence
ASTKGPSVFPLAPSSKSTSGGTAALGCLVKDYFPEPVTVSWNSGALTSGVHTFPAVLQSSGLYSLSSVVTVPSSNFGTQTYTCNVDHKPSNTKVDKTVERKSCVECPPCPAPPVAGPSVFLFPPKPKDTLMISRTPEVTCVVVDVSQEDPEVQFNWYVDGVEVHNAKTKPREEQFNSTFRVVSVLTVVHQDWLNGKEYKCKVSNKGLPAPIEKTISKTKGQPREPQVYTLPPSQEEMTKNQVSLTCLVKGFYPSDIAVEWESNGQPENNYKTTPPMLDSDGSFFLYSKLTVDKSRWQEGNVFSCSVMHEALHNHYTQKSLSLSP

SEQ ID NO: 13 - protein, 326 aa, Artificial
  An artificially synthesized peptide sequence
ASTKGPSVFPLAPCSRSTSESTAALGCLVKDYFPEPVTVSWNSGALTSGVHTFPAVLQSSGLYSLSSVVTVPSSNFGTQTYTCNVDHKPSNTKVDKTVERKCCVECPPCPAPPVAGPSVFLFPPKPKDTLMISRTPEVTCVVVDVSHEDPEVQFNWYVDGVEVHNAKTKPREEQFNSTFRVVSVLTVVHQDWLNGKEYKCKVSNKGLPAPIEKTISKTKGQPREPQVYTLPPSREEMTKNQVSLTCLVKGFYPSDIAVEWESNGQPENNYKTTPPMLDSDGSFFLYSKLTVDKSRWQQGNVFSCSVMHEALHAHYTQKSLSLSPGK

SEQ ID NO: 14 - protein, 324 aa, Artificial
  An artificially synthesized peptide sequence
ASTKGPSVFPLAPSSKSTSGGTAALGCLVKDYFPEPVTVSWNSGALTSGVHTFPAVLQSSGLYSLSSVVTVPSSNFGTQTYTCNVDHKPSNTKVDKTVERKSCVECPPCPAPPVAGPSVFLFPPKPKDTLMISRTPEVTCVVVDVSQEDPEVQFNWYVDGVEVHNAKTKPREEQFNSTFRVVSVLTVVHQDWLNGKEYKCKVSNKGLPAPIEKTISKTKGQPREPQVYTLPPSQEEMTKNQVSLTCLVKGFYPSDIAVEWESNGQPENNYKTTPPMLDSDGSFFLYSKLTVDKSRWQEGNVFSCSVMHEALHAHYTQKSLSLSP

SEQ ID NO: 15 - protein, 443 aa, Artificial
  An artificially synthesized peptide sequence
QVQLQESGPGLVKPSETLSLTCAVSGHSISHDHAWSWVRQPPGEGLEWIGFISYSGITNYNPSLQGRVTISRDNSKNTLYLQMNSLRAEDTAVYYCARSLARTTAMDYWGEGTLVTVSSASTKGPSVFPLAPSSKSTSGGTAALGCLVKDYFPEPVTVSWNSGALTSGVHTFPAVLQSSGLYSLSSVVTVPSSNFGTQTYTCNVDHKPSNTKVDKTVERKSCVECPPCPAPPVAGPSVFLFPPKPKDTLMISRTPEVTCVVVDVSQEDPEVQFNWYVDGVEVHNAKTKPREEQFNSTFRVVSVLTVVHQDWLNGKEYKCKVSNKGLPAPIEKTISKTKGQPREPQVYTLPPSQEEMTKNQVSLTCLVKGFYPSDIAVEWESNGQPENNYKTTPPMLDSDGSFFLYSKLTVDKSRWQEGNVFSCSVMHEALHAHYTQKSLSLSP

SEQ ID NO: 16 - protein, 447 aa, Artificial
  An artificially synthesized peptide sequence
EVQLVESGGKLLKPGGSLKLSCAASGFTFSSFAMSWFRQSPEKRLEWVAEISSGGSYTYYPDTVTGRFTISRDNAKNTLYLEMSSLRSEDTAMYYCARGLWGYYALDYWGQGTSVTVSSASTKGPSVFPLAPSSKSTSGGTAALGCLVKDYFPEPVTVSWNSGALTSGVHTFPAVLQSSGLYSLSSVVTVPSSSLGTQTYICNVNHKPSNTKVDKKVEPKSCDKTHTCPPCPAPELLGGPSVFLFPPKPKDTLMISRTPEVTCVVVDVSHEDPEVKFNWYVDGVEVHNAKTKPREEQYNSTYRVVSVLTVLHQDWLNGKEYKCKVSNKALPAPIEKTISKAKGQPREPQVYTLPPSRDELTKNQVSLTCLVKGFYPSDIAVEWESNGQPENNYKTTPPVLDSDGSFFLYSKLTVDKSRWQQGNVFSCSVMHEALHNHYTQKSLSLSP

SEQ ID NO: 17 - protein, 213 aa, Artificial
  An artificially synthesized peptide sequence
QIVLIQSPAIMSASPGEKVTMTCSASSSVSYMYWYQQKPGSSPRLLIYDTSNLASGVPVRFSGSGSGTSYSLTISRMEAEDAATYYCQQWSGYPYTFGGGTKLEIKRTVAAPSVFIFPPSDEQLKSGTASVVCLLNNFYPREAKVQWKVDNALQSGNSQESVTEQDSKDSTYSLSSTLTLSKADYEKHKVYACEVTHQGLSSPVTKSFNRGEC

SEQ ID NO: 18 - protein, 447 aa, Artificial
  An artificially synthesized peptide sequence
EVQLVESGGKLLKPGGSLKLSCAASGFTFSSHAMSWFRQSPEKRLEWVAEISSGGSYTYHPHTVTGRFTISRDNAKNTLYLEMSSLRSEDTAMYYCARGLWGHYALDYWGQGTSVTVSSASTKGPSVFPLAPSSKSTSGGTAALGCLVKDYFPEPVTVSWNSGALTSGVHTFPAVLQSSGLYSLSSVVTVPSSSLGTQTYICNVNHKPSNTKVDKKVEPKSCDKTHTCPPCPAPELLGGPSVFLFPPKPKDTLMISRTPEVTCVVVDVSHEDPEVKFNWYVDGVEVHNAKTKPREEQYNSTYRVVSVLTVLHQDWLNGKEYKCKVSNKALPAPIEKTISKAKGQPREPQVYTLPPSRDELTKNQVSLTCLVKGFYPSDIAVEWESNGQPENNYKTTPPVLDSDGSFFLYSKLTVDKSRWQQGNVFSCSVMHEALHNHYTQKSLSLSP

SEQ ID NO: 19 - protein, 213 aa, Artificial
  An artificially synthesized peptide sequence
QIVLIQSPAIMSASPGEKVTMTCSASSSVSYMYWYQQKPGSSPRLLIYDTSHHASGVPVRFSGSGSGTSYSLTISRMEAEDAATYYCHQWSGHPYTFGGGTKLEIKRTVAAPSVFIFPPSDEQLKSGTASVVCLLNNFYPREAKVQWKVDNALQSGNSQESVTEQDSKDSTYSLSSTLTLSKADYEKHKVYACEVTHQGLSSPVTKSFNRGEC

SEQ ID NO: 20 - protein, 447 aa, Artificial
  An artificially synthesized peptide sequence
EVQLVESGGKLLKPGGSLKLSCAASGFTFSSHAMSWFRQSPEKRLEWVAEISSGGSYTYHPHTVTGRFTISRDNAKNTLYLEMSSLRSEDTAMYYCARGLWGHYALDYWGQGTSVTVSSASTKGPSVFPLAPSSKSTSGGTAALGCLVKDYFPEPVTVSWNSGALTSGVHTFPAVLQSSGLYSLSSVVTVPSSSLGTQTYICNVNHKPSNTKVDKKVEPKSCDKTHTCPPCPAPELLGGPSVFLFPPKPKDTLMISRTPEVTCVVVDVSHEDPEVKFNWYVDGVEVHNAKTKPREEQYNSTYRVVSVLTVLHQDWLNGKEYKCKVSNKALPAPIEKTISKAKGQPREPQVYTLPPSRDELTKNQVSLTCLVKGFYPSDIAVEWESNGQPENNYKTTPPVLDSDGSFFLYSKLTVDKSRWQQGNVFSCSVMHEALHWHYTQKSLSLSP

SEQ ID NO: 21 - protein, 447 aa, Artificial
  An artificially synthesized peptide sequence
EVQLVESGGKLLKPGGSLKLSCAASGFTFSSHAMSWFRQSPEKRLEWVAEISSGGSYTYHPHTVTGRFTISRDNAKNTLYLEMSSLRSEDTAMYYCARGLWGHYALDYWGQGTSVTVSSASTKGPSVFPLAPSSKSTSGGTAALGCLVKDYFPEPVTVSWNSGALTSGVHTFPAVLQSSGLYSLSSVVTVPSSSLGTQTYICNVNHKPSNTKVDKKVEPKSCDKTHTCPPCPAPELLGGPSVFLFPPKPKDTLWISRTPEVTCVVVDVSHEDPEVKFNWYVDGVEVHNAKTKPREEQYNSTYRVVSVLTVLHQDWLNGKEYKCKVSNKALPAPIEKTISKAKGQPREPQVYTLPPSRDELTKNQVSLTCLVKGFYPSDIAVEWESNGQPENNYKTTPPVLDSDGSFFLYSKLTVDKSRWQQGNVFSCSVMHEALHWHYTQKSLSLSP

SEQ ID NO: 22 - protein, 436 aa, Artificial
  An artificially synthesized peptide sequence
QEGDFPMPFISAKSSPVIPLDGSVKIQCQAIREAYLTQLMIIKNSTYREIGRRLKFWNETDPEFVIDHMDANKAGRYQCQYRIGHYRFRYSDTLELVVTGLYGKPFLSADRGLVLMPGENISLTCSSAHIPFDRFSLAKEGELSLPQHQSGEHPANFSLGPVDLNVSGIYRCYGWYNRSPYLWSFPSNALELVVTGGGGSGGGGSGGGGSGGGGSHTSPPSPAPELLGGPSVFLFPPKPKDTLMISRTPEVTCVVVDVSHEDPEVKFNWYVDGVEVHNAKTKPREEQYNSTYRVVSVLTVLHQDWLNGKEYKCKVSNKALPAPIEKTISKAKGQPREPQVYTLPPSRDELTKNQVSLTCLVKGFYPSDIAVEWESNGQPENNYKTTPPVLDSDGSFFLYSKLTVDKSRWQQGNVFSCSVMHEALHNHYTQKSLSLS

SEQ ID NO: 23 - protein, 436 aa, Artificial [sequence omitted]

SEQ ID NO: 24 - protein, 448 aa, Artificial
  An artificially synthesized peptide sequence
QSLEESGGDLVKPGASLTLTCTASGFSFSSNYWIYWVRQAPGKGLEWIACIYIGSDSAYYASWAKGRFTISKTSSTTVTLQMTSLTAADTATYFCARWDNSGRALKLWGPGTLVTVSSASTKGPSVFPLAPSSKSTSGGTAALGCLVKDYFPEPVTVSWNSGALTSGVHTFPAVLQSSGLYSLSSVVTVPSSSLGTQTYICNVNHKPSNTKVDKKVEPKSCDKTHTCPPCPAPELLGGPSVFLFPPKPKDTLMISRTPEVTCVVVDVSHEDPEVKFNWYVDGVEVHNAKTKPREEQYNSTYRVVSVLTVLHQDWLNGKEYKCKVSNKALPAPIEKTISKAKGQPREPQVYTLPPSRDELTKNQVSLTCLVKGFYPSDIAVEWESNGQPENNYKTTPPVLDSDGSFFLYSKLTVDKSRWQQGNVFSCSVMHEALHNHYTQKSLSLSPGK

SEQ ID NO: 25 - protein, 219 aa, Artificial
  An artificially synthesized peptide sequence
QMLTQTASPVSAAVGGTVTIKCQSSQSVADNNHLSWYQQKPGQPPKLLIYFASTLASGVSSRFKGSGSGTQFTLTISDVQCDDAATYYCLGNYDCGSADCHAFGGGTEVVVKRTVAAPSVFIFPPSDEQLKSGTASVVCLLNNFYPREAKVQWKVDNALQSGNSQESVTEQDSKDSTYSLSSTLTLSKADYEKHKVYACEVTHQGLSSPVTKSFNRGEC

SEQ ID NO: 26 - protein, 454 aa, Artificial
  An artificially synthesized peptide sequence
QEQLEESGGGLVKPEGSLTLTCKASGFDFSSYYYMCWVRQAPGKGLEWIGCIVTGSYGRSWYASWAKGRFTITRSTSLNTVTLQLNSLTAADTATYFCARDPFVIASSHYQNLWGPGTLVTVSSASTKGPSVFPLAPSSKSTSGGTAALGCLVKDYFPEPVTVSWNSGALTSGVHTFPAVLQSSGLYSLSSVVTVPSSSLGTQTYICNVNHKPSNTKVDKKVEPKSCDKTHTCPPCPAPELLGGPSVFLFPPKPKDTLMISRTPEVTCVVVDVSHEDPEVKFNWYVDGVEVHNAKTKPREEQYNSTYRVVSVLTVLHQDWLNGKEYKCKVSNKALPAPIEKTISKAKGQPREPQVYTLPPSRDELTKNQVSLTCLVKGFYPSDIAVEWESNGQPENNYKTTPPVLDSDGSFFLYSKLTVDKSRWQQGNVFSCSVMHEALHNHYTQKSLSLSPGK

SEQ ID NO: 27 - protein, 218 aa, Artificial
  An artificially synthesized peptide sequence
ALVMTQTPSPVSAAVGGTVTISCQSSPNIYNNYLSWYQQKPGQPPKLLIYRASNLETGVPSRFSGSGSGTQFTLTISDVQCDDAATYYCAGYKSYDNDDNAFGGGTEVVVKRTVAAPSVFIFPPSDEQLKSGTASVVCLLNNFYPREAKVQWKVDNALQSGNSQESVTEQDSKDSTYSLSSTLTLSKADYEKHKVYACEVTHQGLSSPVTKSFNRGEC

SEQ ID NO: 28 - protein, 454 aa, Artificial
  An artificially synthesized peptide sequence
QEQLEESGGGLVKPEGSLTLTCKASGFDFSSYYYMCWVRQAPGKGLEWIGCIVTGSYGRSWYASWAKGRFTITRSTSLNTVTLQLNSLTAADTATYFCARDPFVIASSHYQNLWGPGTLVTVSSASTKGPSVFPLAPSSKSTSGGTAALGCLVKDYFPEPVTVSWNSGALTSGVHTFPAVLQSSGLYSLSSVVTVPSSSLGTQTYICNVNHKPSNTKVDKKVEPKSCDKTHTCPPCPAPELLGGPSVFLFPPKPKDTLMISRTPEVTCVVVDVSHEDPEVKFNWYVDGVEVHNAKTKPREEQYNSTYRVVSVLTVLHQDWLNGKEYKCKVSNKALPAPIEKTISKAKGQPREPQVYTLPPSRDELTKNQVSLTCLVKGFYPSDIAVEWESNGQPENNYKTTPPVLDSDGSFFLYSKLTVDKSRWQQGNVFSCSVMHEALHWHYTQKSLSLSPGK

SEQ ID NO: 29 - protein, 472 aa, Artificial
  An artificially synthesized peptide sequence
QVQLQESGPGLVRPSQTLSLTCTVSGYSITSDHAWSWVRQPPGRGLEWIGYISYSGITTYNPSLKSRVTMLRDTSKNQFSLRLSSVTAADTAVYYCARSLARTTAMDYWGQGSLVTVSSASPTSPKVFPLSLCSTQPDGNVVIACLVQGFFPQEPLSVTWSESGQGVTARNFPPSQDASGDLYTTSSQLTLPATQCLAGKSVTCHVKHYTNPSQDVTVPCPVPSTPPTPSPSTPPTPSPSCCHPRLSLHRPALEDLLLGSEANLTCTLTGLRDASGVTFTWTPSSGKSAVQGPPERDLCGCYSVSSVLPGCAEPWNHGKTFTCTAAYPESKTPLTATLSKSGNTFRPEVHLLPPPSEELALNELVTLTCLARGFSPKDVLVRWLQGSQELPREKYLTWASRQEPSQGTTTFAVTSILRVAAEDWKKGDTFSCMVGHEALPLAFTQKTIDRLAGKPTHVNVSVVMAEVDGTCY

SEQ ID NO: 30 - protein, 365 aa, Homo sapiens
MGVPRPQPWALGLLLFLLPGSLGAESHLSLLYHLTAVSSPAPGTPAFWVSGWLGPQQYLSYNSLRGEAEPCGAWVWENQVSWYWEKETTDLRIKEKLFLEAFKALGGKGPYTLQGLLGCELGPDNTSVPTAKFALNGEEFMNFDLKQGTWGGDWPEALAISQRWQQQDKAANKELTFLLFSCPHRLREHLERGRGNLEWKEPPSMRLKARPSSPGFSVLTCSAFSFYPPELQLRFLRNGLAAGTGQGDFGPNSDGSFHASSSLTVKSGDEHHYCCIVQHAGLAQPLRVELESPAKSSVLVVGIVIGVLLLTAAAVGGALLWRRMRSGLPAPWISLRGDDTGVLLPTPGEAQDADLKDVNVIPATA

SEQ ID NO: 31 - protein, 119 aa, Homo sapiens
MSRSVALAVLALLSLSGLEAIQRTPKIQVYSRHPAENGKSNFLNCYVSGFHPSDIEVDLLKNGERIEKVEHSDLSFSKDWSFYLLYYTEFTPTEKDEYACRVNHVTLSQPKIVKWDRDM